European Patent Application EP 4 512 415 A1, published February 26, 2025. Title: CAR for treatment of MS or AD. Applicant: Medizinische Hochschule Hannover. The sequence listing filed with the application follows.

SEQUENCE LISTING (68 sequences)

SEQ ID NO: 1 - protein, 22 aa, synthetic construct
MDFQVQIFSFLLISASVIMSRT

SEQ ID NO: 2 - protein, 21 aa, synthetic construct
MWWRLWWLLLLLLLLWPMVWA

SEQ ID NO: 3 - protein, 20 aa, synthetic construct
MWWRLWWLLLLLLLLWPMVW

SEQ ID NO: 4 - protein, 21 aa, synthetic construct
MDFQVQIFSFLLISASVIMSR

SEQ ID NO: 5 - protein, 226 aa, synthetic construct
VPRDGGCKPCICTVPEVSSVFIFPPKPKDVLTITLTPKVTCVVVDISKDDPEVQFSWFVDDVEVHTAQTQPREEQFNSTFRSVSELPIMHQDWLNGKEFKCRVNSAAFPAPIEKTISKTKGRPKAPQVCTIPPPKEQMAKDKVSLTCMITDFFPEDITVEWQWNGQPAENYKNTQPIMDTDGSYFVYSKLNVQKSNWEAGNTFTCSVLHEGLHNHHTEKSLSHSPG

SEQ ID NO: 6 - protein, 57 aa, synthetic construct
SSVVPVLQKVNSTTTKPVLRTPSPVHPTGTSQPQRPEDCRPRGSVKGTGLDFACDIY

SEQ ID NO: 7 - protein, 83 aa, synthetic construct
FVPVFLPAKPTTTPAPRPPTPAPTIASQPLSLRPEASRPAAGGAVHTRGLDFADIYIWAPLAGTCGVLLLSLVITLYCNHRQL

SEQ ID NO: 8 - protein, 234 aa, synthetic construct
PAEPKSPDKTHTCPPCPAPPVAGPSVFLFPPKPKDTLMIARTPEVTCVVVDVSHEDPEVKFNWYVDGVEVHNAKTKPREEQYNSTYRVVSVLTVLHQDWLNGKEYKCKVSNKALPAPIEKTISKAKGQPREPQVYTLPPSRDELTKNQVSLTCLVKGFYPSDIAVEWESNGQPENNYKTTPPVLDSDGSFFLYSKLTVDKSRWQQGNVFSCSVMHEALHNHYTQKSLSLSPGKK

SEQ ID NO: 9 - protein, 25 aa, synthetic construct
VFLACVLGGSFGFLGFLGLCILCCV

SEQ ID NO: 10 - protein, 25 aa, synthetic construct
IWAPLAGICVALLLSLIITLICYHR

SEQ ID NO: 11 - protein, 42 aa, synthetic construct
NSRRNRLLQSDYMNMTPRRPGLTRKPYQPYAPARDFAAYRPL

SEQ ID NO: 12 - protein, 113 aa, synthetic construct
RAKFSRSAETAANLQDPNQLYNELNLGRREEYDVLEKKRARDPEMGGKQQRRRNPQEGVYNALQKDKMAEAYSEIGTKGERRRGKGHDGLYQGLSTATKDTYDALHMQTLAPR

SEQ ID NO: 13 - protein, 43 aa, synthetic construct
WTNSRRNRLLQSDYMNMTPRRPGLTRKPYQPYAPARDFAAYRP

SEQ ID NO: 14 - protein, 113 aa, synthetic construct; identical to SEQ ID NO: 12

SEQ ID NO: 15 - protein, 42 aa, synthetic construct
VRSKRSRLLHSDYMNMTPRRPGPTRKHYQPYAPPRDFAAYRS

SEQ ID NO: 16 - protein, 115 aa, synthetic construct
RVKFSRSADAPAYQQGQNQLYNELNLGRREEYDVLDKRRGRDPEMGGKPRRKNPQEGLYNELQKDKMAEAYSEIGMKGERRRGKGHDGLYQGLSTATKDTYDALHMQALPPRSSR

SEQ ID NO: 17 - protein, 72 aa, synthetic construct
DPKFWVLVVVGGVLACYSLLVTVAFIIFWVRSKRSRLLHSDYMNMTPRRPGPTRKHYQAYAAARDFAAYRSL

SEQ ID NO: 18 - protein, 112 aa, synthetic construct
RVKFSRSADAPAYQQGQNQLYNELNLGRREEYDVLDKRRGRDPEMGGKPRRKNPQEGLYNELQKDKMAEAYSEIGMKGERRRGKGHDGLYQGLSTATKDTYDALHMQALPPR

SEQ ID NO: 19 - protein, 19 aa, synthetic construct
ATNFSLLKQAGDVEENPGP

SEQ ID NO: 20 - protein, 429 aa, synthetic construct
MPNPRPAKPMAPSLALGPSPGVLPSWKTAPKGSELLGTRGSGGPFQGRDLRSGAHTSSSLNPLPPSQLQLPTVPLVMVAPSGARLGPSPHLQALLQDRPHFMHQLSTVDAHAQTPVLQVRPLDNPAMISLPPPSAATGVFSLKARPGLPPGINVASLEWVSREPALLCTFPRSGTPRKDSNLLAAPQGSYPLLANGVCKWPGCEKVFEEPEEFLKHCQADHLLDEKGKAQCLLQREVVQSLEQQLELEKEKLGAMQAHLAGKMALAKAPSVASMDKSSCCIVATSTQGSVLPAWSAPREAPDGGLFAVRRHLWGSHGNSSFPEFFHNMDYFKYHNMRPPFTYATLIRWAILEAPERQRTLNEIYHWFTRMFAYFRNHPATWKNAIRHNLSLHKCFVRVESEKGAVWTVDEFEFRKKRSQRPNKCSNPCP

SEQ ID NO: 21 - protein, 449 aa, synthetic construct
ATNFSLLKQAGDVEENPGPSMPNPRPAKPMAPSLALGPSPGVLPSWKTAPKGSELLGTRGSGGPFQGRDLRSGAHTSSSLNPLPPSQLQLPTVPLVMVAPSGARLGPSPHLQALLQDRPHFMHQLSTVDAHAQTPVLQVRPLDNPAMISLPPPSAATGVFSLKARPGLPPGINVASLEWVSREPALLCTFPRSGTPRKDSNLLAAPQGSYPLLANGVCKWPGCEKVFEEPEEFLKHCQADHLLDEKGKAQCLLQREVVQSLEQQLELEKEKLGAMQAHLAGKMALAKAPSVASMDKSSCCIVATSTQGSVLPAWSAPREAPDGGLFAVRRHLWGSHGNSSFPEFFHNMDYFKYHNMRPPFTYATLIRWAILEAPERQRTLNEIYHWFTRMFAYFRNHPATWKNAIRHNLSLHKCFVRVESEKGAVWTVDEFEFRKKRSQRPNKCSNPCP

SEQ ID NO: 22 - protein, 431 aa, synthetic construct
MPNPRPGKPSAPSLALGPSPGASPSWRAAPKASDLLGARGPGGTFQGRDLRGGAHASSSSLNPMPPSQLQLPTLPLVMVAPSGARLGPLPHLQALLQDRPHFMHQLSTVDAHARTPVLQVHPLESPAMISLTPPTTATGVFSLKARPGLPPGINVASLEWVSREPALLCTFPNPSAPRKDSTLSAVPQSSYPLLANGVCKWPGCEKVFEEPEDFLKHCQADHLLDEKGRAQCLLQREMVQSLEQQLVLEKEKLSAMQAHLAGKMALTKASSVASSDKGSCCIVAAGSQGPVVPAWSGPREAPDSLFAVRRHLWGSHGNSTFPEFLHNMDYFKFHNMRPPFTYATLIRWAILEAPEKQRTLNEIYHWFTRMFAFFRNHPATWKNAIRHNLSLHKCFVRVESEKGAVWTVDELEFRKKRSQRPSRCSNPTPGP

SEQ ID NO: 23 - DNA, 843 bp, synthetic construct
  source 1..843: mol_type = other DNA
  CDS 1..843: note = LNGFR; protein_id = 24; translation = MGAGATGRAMDGPRLLLLLLLGVSLGGAKEACPTGLYTHSGECCKACNLGEGVAQPCGANQTVCEPCLDSVTFSDVVSATEPCKPCTECVGLQSMSAPCVEADDAVCRCAYGYYQDETTGRCEACRVCEAGSGLVFSCQDKQNTVCEECPDGTYSDEANHVDPCLPCTVCEDTERQLRECTRWADAECEEIPGRWITRSTPPEGSDSTAPSTQEPEAPPEQDLIASTVAGVVTTVMGSSQPVVTRGTTDNLIPVYCSILAAVVVGLVAYIAFKRWNRGIL
atgggcgctggcgccacaggcagagctatggatggacctagactgctcctcctgctgctcctgggagtttctctcggcggagccaaagaggcctgtcctaccggactgtacacacactctggcgagtgctgcaaggcctgcaatctcggagaaggcgtggcacaaccttgcggcgctaatcagaccgtgtgcgagccttgtctggactccgtgacctttagcgacgtggtgtctgccaccgagccttgcaagccttgtaccgagtgtgtgggcctgcagagcatgtctgccccttgtgtggaagccgacgatgccgtgtgtagatgcgcctacggctactaccaggacgagacaacaggcagatgcgaggcctgtagagtgtgcgaagctggctctggactggtgttcagctgccaagacaagcagaacaccgtgtgtgaagagtgccccgacggcacctatagcgacgaagccaatcacgtggacccctgcctgccttgtactgtgtgcgaggacaccgagcggcagctgagagaatgtactagatgggccgacgccgagtgcgaagagatccctggaagatggatcaccagaagcaccccacctgagggcagcgattctacagccccaagcacacaagagcccgaggctcctccagaacaggacctgattgcctctacagtggccggcgtcgtgacaacagtgatgggatcttctcagcccgtggtcaccaggggcaccaccgataatctgatccccgtgtactgcagcatcctggccgctgtggttgtgggactcgtggcctatatcgccttcaagcggtggaaccggggcatcctctaa

SEQ ID NO: 24 - protein, 280 aa, synthetic construct
MGAGATGRAMDGPRLLLLLLLGVSLGGAKEACPTGLYTHSGECCKACNLGEGVAQPCGANQTVCEPCLDSVTFSDVVSATEPCKPCTECVGLQSMSAPCVEADDAVCRCAYGYYQDETTGRCEACRVCEAGSGLVFSCQDKQNTVCEECPDGTYSDEANHVDPCLPCTVCEDTERQLRECTRWADAECEEIPGRWITRSTPPEGSDSTAPSTQEPEAPPEQDLIASTVAGVVTTVMGSSQPVVTRGTTDNLIPVYCSILAAVVVGLVAYIAFKRWNRGIL

SEQ ID NO: 25 - DNA, 786 bp, synthetic construct
  source 1..786: mol_type = other DNA; note = scFv SH1990-C1
  CDS 1..786: protein_id = 26; translation = MAQVQLQESGGGLVKPGGSLRLSCAASGFTFSDYYMSWIRQAPGKGLEWVSYISSSGSTIYYADSVKGRFTISRDNAKNSLYLQMNSLRAEDTAVYYCARGGGDFDYWGQGTLVTVSSGSASAPKLEEGEFSEARVNFMLTQPHSVSESPGKTVTISCTGSSGSIASSYVQWYQQRPGSAPTTVIFEDYRRPSGVPDRFSGSVDRSSNSASLTISGLKIEDEADYYCQSYGSTDVVFGGGTKLTVLSQPKAAPSVTLFPPSS
atggcccaggtgcagctgcaggagtcggggggaggcttggtcaagcctggagggtccctgagactctcctgtgcagcctctggattcaccttcagtgactactacatgagctggatccgccaggctccagggaaggggctggagtgggtttcatacattagtagtagtggtagtaccatatactacgcagactctgtgaagggccgattcaccatctccagggacaacgccaagaactcactgtatctgcaaatgaacagcctgagagccgaggacacggccgtgtattactgtgcgagagggggcggagactttgactactggggccagggaaccctggtcaccgtctcctcagggagtgcatccgccccaaagcttgaagaaggtgaattttcagaagcacgcgtaaattttatgctgactcagccccactctgtgtcggagtctccggggaagacggtaaccatctcctgcaccggcagcagtggcagcattgccagcagctatgtgcagtggtaccagcagcgcccgggcagtgcccccaccactgtgatctttgaggattaccgaagaccgtctggggtccctgatcggttctctggctccgtcgacaggtcttccaactctgcctccctcaccatctctggactgaagattgaggacgaggctgactattactgtcagtcttatggtagcaccgatgtggtattcggcggagggaccaagctgaccgtcctgagtcagcccaaggctgccccctcggtcactctgttcccaccctcctct

SEQ ID NO: 26 - protein, 262 aa, synthetic construct
MAQVQLQESGGGLVKPGGSLRLSCAASGFTFSDYYMSWIRQAPGKGLEWVSYISSSGSTIYYADSVKGRFTISRDNAKNSLYLQMNSLRAEDTAVYYCARGGGDFDYWGQGTLVTVSSGSASAPKLEEGEFSEARVNFMLTQPHSVSESPGKTVTISCTGSSGSIASSYVQWYQQRPGSAPTTVIFEDYRRPSGVPDRFSGSVDRSSNSASLTISGLKIEDEADYYCQSYGSTDVVFGGGTKLTVLSQPKAAPSVTLFPPSS

SEQ ID NO: 27 - DNA, 804 bp, synthetic construct
  source 1..804: mol_type = other DNA
  CDS 1..804: note = scFv SH1990-C3; protein_id = 28; translation = MAQVQLQQSGAEVKKPGASVKVSCKASGYTFTSYYMHWVRQAPGQGLEWMGIINPSGGSTSYAQKFQGRVTMTRDTSTSTVYMELSSLRSEDTAVYYCARESVVRGVNLSFDYWGQGTLVTVSSGSASAPKLEEGEFSEARVLPVLTQPPSASGTPGQRVTISCSGSSSNIGSNYAYWYQQLPGTAPKLLIYSNNQRPSGVPDRFSGSKSGTSASLAISGLQSEDEADYYCAAWDDSLNGVVFGGGTKLTVLGQPKAAPSVTLFPPSS
atggcccaggtacagctgcagcagtcaggggctgaggtgaagaagcctggggcctcagtgaaggtttcctgcaaggcatctggatacaccttcaccagctactatatgcactgggtgcgacaggcccctggacaagggcttgagtggatgggaataatcaaccctagtggtggtagcacaagctacgcacagaagttccagggcagagtcaccatgaccagggacacgtccacgagcacagtctacatggagctgagcagcctgagatctgaggacacggccgtgtattactgtgcgagagagtcggtggttcggggagttaacctaagttttgactactggggccagggaaccctggtcaccgtctcctcagggagtgcatccgccccaaagcttgaagaaggtgaattttcagaagcacgcgtactgcctgtgctgactcagcccccctcagcgtctgggacccccgggcagagggtcaccatctcttgttctggaagcagctccaacatcggaagtaattatgcatactggtaccagcagctcccaggaacggcccccaaactcctcatctatagtaataatcagcggccctcaggggtccctgaccgattctctggctccaagtctggcacctcagcctccctggccatcagtgggctccagtctgaggatgaggctgattattactgtgcagcatgggatgacagcctgaatggggtggtattcggcggagggaccaagctgaccgtcctaggtcagcccaaggctgccccctcggtcactctgttcccgccctcctct

SEQ ID NO: 28 - protein, 268 aa, synthetic construct
MAQVQLQQSGAEVKKPGASVKVSCKASGYTFTSYYMHWVRQAPGQGLEWMGIINPSGGSTSYAQKFQGRVTMTRDTSTSTVYMELSSLRSEDTAVYYCARESVVRGVNLSFDYWGQGTLVTVSSGSASAPKLEEGEFSEARVLPVLTQPPSASGTPGQRVTISCSGSSSNIGSNYAYWYQQLPGTAPKLLIYSNNQRPSGVPDRFSGSKSGTSASLAISGLQSEDEADYYCAAWDDSLNGVVFGGGTKLTVLGQPKAAPSVTLFPPSS

SEQ ID NO: 29 - protein, 116 aa, synthetic construct
  source 1..116: note = VH of scFv SH1990-C1
  CHAIN 26..33: note = CDR1
  CHAIN 51..58: note = CDR2
  CHAIN 97..105: note = CDR3
QVQLQESGGGLVKPGGSLRLSCAASGFTFSDYYMSWIRQAPGKGLEWVSYISSSGSTIYYADSVKGRFTISRDNAKNSLYLQMNSLRAEDTAVYYCARGGGDFDYWGQGTLVTVSS

SEQ ID NO: 30 - protein, 110 aa, synthetic construct
  source 1..110: note = VL of scFv SH1990-C1
  CHAIN 26..33: note = CDR1
  CHAIN 51..53: note = CDR2
  CHAIN 92..100: note = CDR3
NFMLTQPHSVSESPGKTVTISCTGSSGSIASSYVQWYQQRPGSAPTTVIFEDYRRPSGVPDRFSGSVDRSSNSASLTISGLKIEDEADYYCQSYGSTDVVFGGGTKLTVL

SEQ ID NO: 31 - protein, 122 aa, synthetic construct
  source 1..122: note = VH of scFv SH1990-C3
  CHAIN 26..33: note = CDR1
  CHAIN 51..58: note = CDR2
  CHAIN 97..111: note = CDR3
QVQLQQSGAEVKKPGASVKVSCKASGYTFTSYYMHWVRQAPGQGLEWMGIINPSGGSTSYAQKFQGRVTMTRDTSTSTVYMELSSLRSEDTAVYYCARESVVRGVNLSFDYWGQGTLVTVSS

SEQ ID NO: 32 - protein, 110 aa, synthetic construct
  source 1..110: note = VL of scFv SH1990-C3
  CHAIN 26..33: note = CDR1
  CHAIN 51..53: note = CDR2
  CHAIN 90..100: note = CDR3
LPVLTQPPSASGTPGQRVTISCSGSSSNIGSNYAYWYQQLPGTAPKLLIYSNNQRPSGVPDRFSGSKSGTSASLAISGLQSEDEADYYCAAWDDSLNGVVFGGGTKLTVL

SEQ ID NO: 33 - DNA, 804 bp, synthetic construct
  source 1..804: mol_type = other DNA
  CDS 1..804: note = scFv SH1986-B2; protein_id = 34; translation = MAQVQLVQSGGGVVQPGRSLRLSCAASGFTFSSYAMHWVRQAPGKGLEWVAVISYDGSNKYYADSVKGRFTISRDNSKNTLYLQMNSLRAEDTAVYYCARDAGGDSSGPYFDYWGQGTLVTVSSGSASAPKLEEGEFSEARVQSALTQPASVSGSPGQSITISCTGTSSDVGGYNFVSWYQQHPGKAPKLMIYAVSERPSGVSNRFSGSKSGNTASLTISGLQAEDEADYYCSSYRSRDALVFGGGTKLTVLGQPKAAPSVTLFPPSS
atggcccaagtgcagctggtacagtctgggggaggcgtggtccagcctgggaggtccctgagactctcctgtgcagcctctggattcaccttcagtagctatgctatgcactgggtccgccaggctccaggcaaggggctggagtgggtggcagttatatcatatgatggaagcaataaatactacgcagactccgtgaagggccgattcaccatctccagagacaattccaagaacacgctgtatctgcaaatgaacagcctgagagctgaggacacggctgtgtattactgtgcgagagatgccgggggtgatagtagtggtccttactttgactactggggccagggaaccctggtcaccgtctcctcagggagtgcatccgccccaaagcttgaagaaggtgaattttcagaagcacgcgtacagtctgccctgactcagcctgcctccgtgtctgggtctcctggacagtcgatcaccatctcctgcactggaaccagcagtgacgttggtggttataactttgtctcctggtaccagcagcacccaggcaaagcccccaaactcatgatttatgctgtcagtgagcggccctcaggggtttctaatcgcttctctggctccaagtctggcaacacggcctccctgaccatctctgggctccaggctgaggacgaggctgattattactgcagctcatatagaagcagggacgctttggtattcggcggagggaccaagctgaccgtcctaggtcagcccaaggctgccccctcggtcactctgttcccaccctcctct

SEQ ID NO: 34 - protein, 268 aa, synthetic construct
MAQVQLVQSGGGVVQPGRSLRLSCAASGFTFSSYAMHWVRQAPGKGLEWVAVISYDGSNKYYADSVKGRFTISRDNSKNTLYLQMNSLRAEDTAVYYCARDAGGDSSGPYFDYWGQGTLVTVSSGSASAPKLEEGEFSEARVQSALTQPASVSGSPGQSITISCTGTSSDVGGYNFVSWYQQHPGKAPKLMIYAVSERPSGVSNRFSGSKSGNTASLTISGLQAEDEADYYCSSYRSRDALVFGGGTKLTVLGQPKAAPSVTLFPPSS

SEQ ID NO: 35 - DNA, 810 bp, synthetic construct
  source 1..810: mol_type = other DNA
  CDS 1..810: note = scFv SH1986-E3; protein_id = 36; translation = MAQVQLVQSGGGVVQPGTSLRLSCAASGFTFSSYGMHWVRQAPGKGLEWVAVISYDGSNKYYADSVKGRFTISRDNSKNTLYLQMNSLRAEDTAVYYCAKDYSYYYGSGSYFNAFDIWGQGTMVTVSSGSASAPKLEEGEFSEARVSSELTQDPAVSVALGQTVGITCQGDSLRSSFASWYQQKPGQAPILVIYGKNNRPSGIPDRFSGSSSGNTVSLTITGAQAEDEADYYCNSRDSSGNHLVFGGGTKLTVLGQPKAAPSVTLFPPSS
atggcccaggtgcagctggtgcagtctgggggaggcgtggtccagcctgggacgtccctgagactctcctgtgcagcctctggattcaccttcagtagctatggcatgcactgggtccgccaggctccaggcaaggggctggagtgggtggcagttatatcatatgatggaagtaataaatactatgcagactccgtgaagggccgattcaccatctccagagacaattccaagaacacgctgtatctgcaaatgaacagcctgagagctgaggacacggctgtgtattactgtgcgaaagattactcgtattactatggttcagggagttattttaatgcttttgatatctggggccaagggacaatggtcaccgtctcttcagggagtgcatccgccccaaagcttgaagaaggtgaattttcagaagcacgcgtatcttctgagctgactcaggaccctgctgtgtctgtggccttgggacagacagtcgggatcacatgccaaggagacagcctcagaagctcttttgcaagttggtaccagcagaagccaggacaggcccctatacttgtcatctatggtaaaaacaaccggccctcagggatcccagaccgattctctggctccagctcaggaaacacagtttccttgaccatcactggggctcaggcggaagatgaggctgactattactgtaactcccgggacagcagtggtaaccatctggtattcggcggagggaccaagctgaccgtcctaggtcagcccaaggctgccccctcggtcactctgttcccgccctcctct

SEQ ID NO: 36 - protein, 270 aa, synthetic construct
MAQVQLVQSGGGVVQPGTSLRLSCAASGFTFSSYGMHWVRQAPGKGLEWVAVISYDGSNKYYADSVKGRFTISRDNSKNTLYLQMNSLRAEDTAVYYCAKDYSYYYGSGSYFNAFDIWGQGTMVTVSSGSASAPKLEEGEFSEARVSSELTQDPAVSVALGQTVGITCQGDSLRSSFASWYQQKPGQAPILVIYGKNNRPSGIPDRFSGSSSGNTVSLTITGAQAEDEADYYCNSRDSSGNHLVFGGGTKLTVLGQPKAAPSVTLFPPSS

SEQ ID NO: 37 - DNA, 792 bp, synthetic construct
  source 1..792: mol_type = other DNA
  CDS 1..792: note = scFv SH1986-G11; protein_id = 38; translation = MAQVQLVQSGAEVEKPGASVKVSCKVSGYTLTKLSMHWVRQAPGKGLEWMGGFDPEDGETIYAQKFQGRVTMTEDTSTDTAYMELSSLRSEDTAVYYCATDILGYCSSTSCYRDYWGQGTLVTVSSGSASAPKLEEGEFSEARVEVVLTQSPLSLPISLGQPASISCRSSQSLLHSNGYNYLDWYLQKPGQSPQLLIYLGSNRASGVPDRFSGSGSGTDFTLKISRVEAEDVGVYYCMQALQTPRTFGQGTKVEIKRTVAAPSV
atggcccaggttcagctggtgcagtctggggctgaggtggagaagcctggggcctcagtgaaggtctcctgcaaggtttccggatacaccctcactaaattatccatgcactgggtgcgacaggctcctggaaaagggcttgagtggatgggaggttttgatcctgaagatggtgaaacaatctacgcacagaagttccagggcagagtcaccatgaccgaggacacatctacagacacagcctacatggagctgagcagcctgagatctgaggacacggccgtgtattactgtgcaacagatatactaggatattgtagtagtaccagctgctatcgggactactggggccagggaaccctggtcaccgtctcctcagggagtgcatccgccccaaagcttgaagaaggtgaattttcagaagcacgcgtagaagttgtgctgactcagtctccactctccctgcccatcagccttggacagccggcctccatctcctgcaggtctagtcagagcctcctgcatagtaatggatacaactatttggattggtacctgcagaagccagggcagtctccacagctcctgatctatttgggttctaatcgggcctccggggtccctgacaggttcagtggcagtggatcaggcacagattttacactgaaaatcagcagagtggaggctgaggatgttggggtttattactgcatgcaagctctacaaactcctcggacgttcggccaagggaccaaggtggaaatcaaacgaactgtggctgcaccatctgtc

SEQ ID NO: 38 - protein, 264 aa, synthetic construct
MAQVQLVQSGAEVEKPGASVKVSCKVSGYTLTKLSMHWVRQAPGKGLEWMGGFDPEDGETIYAQKFQGRVTMTEDTSTDTAYMELSSLRSEDTAVYYCATDILGYCSSTSCYRDYWGQGTLVTVSSGSASAPKLEEGEFSEARVEVVLTQSPLSLPISLGQPASISCRSSQSLLHSNGYNYLDWYLQKPGQSPQLLIYLGSNRASGVPDRFSGSGSGTDFTLKISRVEAEDVGVYYCMQALQTPRTFGQGTKVEIKRTVAAPSV

SEQ ID NO: 39 - DNA, 795 bp, synthetic construct
  source 1..795: mol_type = other DNA
  CDS 1..795: note = scFv VS002-B5; protein_id = 40; translation = MAQVQLQQSGAEMKKPGASVKVSCKASGYTFTKYYMHWVRQAPGQGLEWMGIIDPSGGSTSYAQSFQGRVTMTRDTSTTTVYMELTSLRSEDTAVYYCARGGVPGHYFNWWGQGTLVTVSSGSASAPKLEEGEFSEARVQLVLTQSSSVSVAPGKTARITCGGNNIGSKSVHWYQQKPGQAPVLVIYYDSDRPSGIPERFSGSNSGNTATLTISRVEAGDEADYYCQVWDSSSDHPDVVFGGGTKLTVLGQPKAAPSVTLFPPSS
atggcccaggtacagctgcagcagtcaggggctgagatgaagaagcctggggcctcagtgaaggtttcctgcaaggcatctggatacaccttcaccaagtactatatgcactgggtgcgacaggcccctggacaagggcttgagtggatgggaataatcgaccccagtggtggcagcacaagctacgcacagagcttccagggcagagtcaccatgaccagggacacgtccacgaccacagtctacatggagctgaccagcctgagatctgaagacacggccgtgtattactgtgcgagagggggggtcccgggccattactttaactggtggggccagggaaccctggtcaccgtctcctcagggagtgcatccgccccaaagcttgaagaaggtgaattttcagaagcacgcgtacagcttgtgctgactcaatcatcctcagtgtcagtggccccaggaaagacggccaggattacctgtgggggaaacaacattggaagtaaaagtgtgcactggtaccagcagaagccaggccaggcccctgtgctggtcatctattatgatagcgaccggccctcagggatccctgagcgattctctggctccaactctgggaacacggccaccctgaccatcagcagggtcgaagccggggatgaggccgactattactgtcaggtgtgggatagtagtagtgatcatccggatgtggtattcggcggagggaccaagctgaccgtcctaggtcagcccaaggctgccccctcggtcactctgttcccaccgtcctct

SEQ ID NO: 40 - protein, 265 aa, synthetic construct
MAQVQLQQSGAEMKKPGASVKVSCKASGYTFTKYYMHWVRQAPGQGLEWMGIIDPSGGSTSYAQSFQGRVTMTRDTSTTTVYMELTSLRSEDTAVYYCARGGVPGHYFNWWGQGTLVTVSSGSASAPKLEEGEFSEARVQLVLTQSSSVSVAPGKTARITCGGNNIGSKSVHWYQQKPGQAPVLVIYYDSDRPSGIPERFSGSNSGNTATLTISRVEAGDEADYYCQVWDSSSDHPDVVFGGGTKLTVLGQPKAAPSVTLFPPSS

SEQ ID NO: 41 - DNA, 798 bp, synthetic construct
  source 1..798: mol_type = other DNA
  CDS 1..798: note = scFv VS002-C4; protein_id = 42; translation = MAQMQLVQSGGGLVQPGGSLRLSCAASGFTFSDYYMDWVRQAPGKGLEWVGRIRNKADSYNIDYAASVTGRFTISRDDSKKSLYLQMNSLKIEDTALYYCARISRFDAFDIWGQGTMVTVSSGSASAPKLEEGEFSEARVQPVLTQPPSASGTPGQRVNISCSGGSSNIGSNHVFWYQQFPGTAPRLVIYRNNQRPSGVPDRFSGSKSGTSASLVISGLRSEDEADYYCAAWDDSLSGWVFGGGTKLTVLGQPKAAPSVTLFPPSS
atggcccaaatgcagctggtgcagtctgggggaggcttggtccagcctggagggtccctgagactctcctgtgcagcctctggattcaccttcagtgactactacatggactgggtccgccaggctccagggaaggggctggagtgggttggccgcatcagaaacaaagctgacagttacaacatagattacgccgcgtctgtgacaggcagattcaccatctcaagagatgattcaaagaagtcactgtatctgcaaatgaacagcctgaaaatcgaggacacggccctgtattattgtgctagaatttcgcgctttgatgcctttgatatctggggccaagggacaatggtcaccgtctcttcagggagtgcatccgccccaaagcttgaagaaggtgaattttcagaagcacgcgtacagcctgtgctgactcagccaccctcagcgtctgggacccccgggcagagggtcaacatctcttgttctggaggcagctccaacatcggaagcaatcatgtattttggtatcaacagttcccaggaacggcccccagactcgtcatctataggaataatcaacggccctcaggggtccctgaccgattctctggttccaagtctggcacctcagcctccctggtcatcagtgggctccggtccgaggatgaggctgattattactgtgcagcatgggatgacagcctgagtggttgggtgttcggcggagggaccaagctgaccgtcctaggtcagcccaaggctgccccctcggtcactctgttcccgccctcctct

SEQ ID NO: 42 - protein, 266 aa, synthetic construct
MAQMQLVQSGGGLVQPGGSLRLSCAASGFTFSDYYMDWVRQAPGKGLEWVGRIRNKADSYNIDYAASVTGRFTISRDDSKKSLYLQMNSLKIEDTALYYCARISRFDAFDIWGQGTMVTVSSGSASAPKLEEGEFSEARVQPVLTQPPSASGTPGQRVNISCSGGSSNIGSNHVFWYQQFPGTAPRLVIYRNNQRPSGVPDRFSGSKSGTSASLVISGLRSEDEADYYCAAWDDSLSGWVFGGGTKLTVLGQPKAAPSVTLFPPSS

SEQ ID NO: 43 - DNA, 798 bp, synthetic construct
  source 1..798: mol_type = other DNA
  CDS 1..798: note = scFv VS002-C5; protein_id = 44; translation = MAQVQLVQSGGGLVQPGGSLRLSCAASGFTFSSYAMSWVRQAPGKGLEWVSAISGSGGSTYYADSVKGRFTISRDNSKNTLYLQMNSLRAEDTAVYYCARGWQLWGIDYWGQGTLVTVSSGSASAPKLEEGEFSEARVLPVLTQPHSVSGSPGKTVTISCTRSSGSIAGNYVHWYQQRPGSAPTTVIYEDNQRPSGVPDRFSGSIDSSSNSASLTISGLKTEDEADYYCQSYDGDVQHVVFGGGTKVTVLGQPKAAPSVTLFPPSS
atggcccaggtgcagctggtgcagtctgggggaggcttggtacagcctggggggtccctgagactctcctgtgcagcctctggattcacctttagcagctatgccatgagctgggtccgccaggctccagggaaggggctggagtgggtctcagctattagtggtagtggtggtagcacatactacgcagactccgtgaagggccggttcaccatctccagagacaattccaagaacacgctgtatctgcaaatgaacagcctgagagccgaggacacggccgtatattactgtgcgagagggtggcagctatggggcattgactactggggccagggaaccctggtcaccgtctcctcagggagtgcatccgccccaaagcttgaagaaggtgaattttcagaagcacgcgtactgcctgtgctgactcagccccactctgtgtcggggtctccggggaagacggtaaccatctcctgcacccgcagcagtggcagcattgccggcaactatgtgcactggtaccagcagcgcccgggcagtgcccccaccactgtgatctatgaggataaccaaagaccctctggggtccctgatcggttctctggctccatcgacagctcctccaactctgcctccctcaccatctctggactgaagactgaggacgaggctgactactactgtcagtcttatgatggcgacgttcaacatgtggtcttcggcggagggaccaaggtgaccgtccttggtcagcccaaggctgccccctcggtcactctgttcccgccctcctct

SEQ ID NO: 44 - protein, 266 aa, synthetic construct
MAQVQLVQSGGGLVQPGGSLRLSCAASGFTFSSYAMSWVRQAPGKGLEWVSAISGSGGSTYYADSVKGRFTISRDNSKNTLYLQMNSLRAEDTAVYYCARGWQLWGIDYWGQGTLVTVSSGSASAPKLEEGEFSEARVLPVLTQPHSVSGSPGKTVTISCTRSSGSIAGNYVHWYQQRPGSAPTTVIYEDNQRPSGVPDRFSGSIDSSSNSASLTISGLKTEDEADYYCQSYDGDVQHVVFGGGTKVTVLGQPKAAPSVTLFPPSS

SEQ ID NO: 45 - DNA, 807 bp, synthetic construct
  source 1..807: mol_type = other DNA
  CDS 1..807: note = scFv VS002-G9; protein_id = 46; translation = MAQVQLVESGGGLVQPGGSLRLSCAASGFTFSSFGMHWVRQAPGKGLEWVSAISGSGGSTYYADSVKGRFTISRDNSKNTLYLQMNSLRAEDTAVYYCAKGAYDYGYYYYGMDVWGQGTTVTVSSGSASAPKLEEGEFSEARVNFMLTQPHSVSESPGKTVTISCTRSSGSIASNYVQWYQQRPGSAPTTVIYEDNQRPSGVPDRFSGSIDSSSNSASLTISGLKTEDEADYYCQSSDSNIEVFGGGTKLTVLGQPKAAPSVTLFPPSS
atggcccaggtgcagctggtggagtctgggggaggcttggtacagcctggggggtccctgagactctcctgtgcagcctctggattcaccttcagcagctttggcatgcactgggtccgccaggctccagggaaggggctggagtgggtctcagctattagtggtagtggtggtagcacatactacgcagactccgtgaagggccggttcaccatctccagagacaattccaagaacacgctgtatctgcaaatgaacagcctgagagccgaggacacggccgtatattactgtgcgaaaggagcctatgactacggctactactactacggtatggacgtctggggccaagggaccacggtcaccgtctcctcagggagtgcatccgccccaaagcttgaagaaggtgaattttcagaagcacgcgtaaattttatgctgactcagccccactctgtgtcggagtctccggggaagacggtaaccatctcctgcacccgcagcagtggcagcattgccagcaactatgtgcagtggtaccagcagcgcccgggcagtgcccccaccactgtgatctatgaggataaccaaagaccctctggggtccctgatcggttctctggctccatcgacagctcctccaactctgcctccctcaccatctctggactgaagactgaggacgaggctgactactactgtcagtcttctgatagcaacatagaagtattcggcggagggaccaaactgaccgtcctgggtcagcccaaggctgccccctcggtcactctgttcccgccctcctct

SEQ ID NO: 46 - protein, 269 aa, synthetic construct
MAQVQLVESGGGLVQPGGSLRLSCAASGFTFSSFGMHWVRQAPGKGLEWVSAISGSGGSTYYADSVKGRFTISRDNSKNTLYLQMNSLRAEDTAVYYCAKGAYDYGYYYYGMDVWGQGTTVTVSSGSASAPKLEEGEFSEARVNFMLTQPHSVSESPGKTVTISCTRSSGSIASNYVQWYQQRPGSAPTTVIYEDNQRPSGVPDRFSGSIDSSSNSASLTISGLKTEDEADYYCQSSDSNIEVFGGGTKLTVLGQPKAAPSVTLFPPSS

SEQ ID NO: 47 - DNA, 918 bp, synthetic construct
  source 1..918: mol_type = other DNA
  CDS 1..918: note = scFv MRU185-C11; protein_id = 48; translation = MKYLLPTAAAGLLLLAAQPAMAEVQLVQSGGGVVQPGRSLRLSCAASGFTFSSYAMHWVRQAPGKGLEWVAVISYDGSNKYYADSVKGRFTISRDNSKNTLYLQMNSLRAEDTAVYYCARGFGGATSYFDYWGQGTLVTVSSGSASAPKLEEGEFSEARVSSELTQDPAVSVALGQTVRITCQGDSLRSYYASWYQQKPGRAPVLVIYGKNNRPSGIPDRFSGSSSGNTASLTITGAQAEDEADYYCNSRDSSGNPVVFGGGTKLTVLGQPKAAPSVTLFPPSSAAAGSEQKLISEEDLSHHHHHH
atgaaatacctattgcctacggcagccgctggcttgctgctgctggcagctcagccggccatggccgaggtgcagctggtgcagtctgggggaggcgtggtccagcctgggaggtccctgagactctcctgtgcagcctctggattcaccttcagtagctatgctatgcactgggtccgccaggctccaggcaaggggctggagtgggtggcagttatatcatatgatggaagtaataaatactacgcagactccgtgaagggccgattcaccatctccagagacaattccaagaacacgctgtatctgcaaatgaacagcctgagagctgaggacacggctgtgtattactgtgcgagagggttcgggggagctactagctactttgactactggggccagggaaccctggtcaccgtctcctcagggagtgcatccgccccaaagcttgaagaaggtgaattttcagaagcacgcgtatcttctgagctgactcaggaccctgctgtgtctgtggccttgggacagacagtcaggatcacatgccaaggagacagcctcagaagctattatgcaagctggtaccagcagaagccaggacgggcccctgtacttgtcatctatggtaaaaacaaccggccctcagggatcccagaccgattctctggctccagctcaggaaacacagcttccttgaccatcactggggctcaggcggaagatgaggctgactattactgtaactcccgggacagcagtggtaaccccgtggtattcggcggagggaccaagctgaccgtcctaggtcagcccaaggctgccccctcggtcactctgttcccaccgtcctctgcggccgcaggttctgaacaaaagctgatctcagaagaagatctatcccatcatcaccatcatcat

SEQ ID NO: 48 - protein, 306 aa, synthetic construct
MKYLLPTAAAGLLLLAAQPAMAEVQLVQSGGGVVQPGRSLRLSCAASGFTFSSYAMHWVRQAPGKGLEWVAVISYDGSNKYYADSVKGRFTISRDNSKNTLYLQMNSLRAEDTAVYYCARGFGGATSYFDYWGQGTLVTVSSGSASAPKLEEGEFSEARVSSELTQDPAVSVALGQTVRITCQGDSLRSYYASWYQQKPGRAPVLVIYGKNNRPSGIPDRFSGSSSGNTASLTITGAQAEDEADYYCNSRDSSGNPVVFGGGTKLTVLGQPKAAPSVTLFPPSSAAAGSEQKLISEEDLSHHHHHH

SEQ ID NO: 49 - DNA, 882 bp, synthetic construct
  source 1..882: mol_type = other DNA
  CDS 1..882: note = scFv MRU185-3-E1; protein_id = 50; translation = MKYLLPTAAAGLLLLAAQPAMAQVQLQESGGGVVQPGRSLRLSCAASGFTFSSYGMHWVRQAPGKGLEWVAVISYDGSKKYYADSVKGRFTISRDNAKNTLYLQMNSLRAEDTAVYYCATGNSHAFDIWGQGTMVTVSSGSASAPKLEEGEFSEARVDIQMTQSPSTLTASVGDRVTVTCRASQTINRWLAWYQQKPGKAPKLLIYLASSLDSGVPSRFSGSGSGTEFTLTISSLQPDDFATYYCQQYNAYPRTFGRGTKVEIKRTVAAPSVAAAGSEQKLISEEDLSHHHHHH
atgaaatacctattgcctacggcagccgctggcttgctgctgctggcagctcagccggccatggcccaggtgcaactgcaggagtcggggggaggcgtggtccagcctgggaggtccctgagactctcctgtgcagcctctggattcaccttcagtagctatggcatgcactgggtccgccaggctccaggcaaggggctggagtgggtggcagttatatcatatgatggaagtaagaaatactatgcagactccgtgaagggccgattcaccatctccagagacaacgccaagaacacgctgtacttgcaaatgaacagtctgagagccgaggacacggctgtatattattgtgctactggtaactctcatgcttttgatatctggggccaagggacaatggtcaccgtctcttcagggagtgcatccgccccaaagcttgaagaaggtgaattttcagaagcacgcgtagacatccagatgacccagtctccatccaccctgactgcatctgttggagacagagtcaccgtcacttgccgggccagtcagactattaataggtggttggcctggtatcagcagaaaccggggaaagcccctaagctcctgatctatctggcgtcttctttagacagtggggtcccatcaaggttcagcggcagtggatctgggacagaattcactctcaccatcagcagcctgcagcctgatgattttgcaacttattactgccaacaatataatgcttatccgaggacgttcggccgagggaccaaggtggaaatcaaacgaactgtggctgcaccatctgtcgcggccgcaggttctgaacaaaagctgatctcagaagaagatctatcccatcatcaccatcatcat

SEQ ID NO: 50 - protein, 294 aa, synthetic construct
MKYLLPTAAAGLLLLAAQPAMAQVQLQESGGGVVQPGRSLRLSCAASGFTFSSYGMHWVRQAPGKGLEWVAVISYDGSKKYYADSVKGRFTISRDNAKNTLYLQMNSLRAEDTAVYYCATGNSHAFDIWGQGTMVTVSSGSASAPKLEEGEFSEARVDIQMTQSPSTLTASVGDRVTVTCRASQTINRWLAWYQQKPGKAPKLLIYLASSLDSGVPSRFSGSGSGTEFTLTISSLQPDDFATYYCQQYNAYPRTFGRGTKVEIKRTVAAPSVAAAGSEQKLISEEDLSHHHHHH

SEQ ID NO: 51 - protein, 122 aa, synthetic construct
  source 1..122: note = VH of scFv SH1986-B2
  CHAIN 26..33: note = CDR1
  CHAIN 51..58: note = CDR2
  CHAIN 97..111: note = CDR3
QVQLVQSGGGVVQPGRSLRLSCAASGFTFSSYAMHWVRQAPGKGLEWVAVISYDGSNKYYADSVKGRFTISRDNSKNTLYLQMNSLRAEDTAVYYCARDAGGDSSGPYFDYWGQGTLVTVSS

SEQ ID NO: 52 - protein, 110 aa, synthetic construct
  source 1..110: note = VL of scFv SH1986-B2
  CHAIN 26..34: note = CDR1
  CHAIN 52..54: note = CDR2
  CHAIN 91..100: note = CDR3
QSALTQPASVSGSPGQSITISCTGTSSDVGGYNFVSWYQQHPGKAPKLMIYAVSERPSGVSNRFSGSKSGNTASLTISGLQAEDEADYYCSSYRSRDALVFGGGTKLTVL

SEQ ID NO: 53 - protein, 126 aa, synthetic construct
  source 1..126: note = VH of scFv SH1986-E3
  CHAIN 26..33: note = CDR1
  CHAIN 51..58: note = CDR2
  CHAIN 97..115: note = CDR3
QVQLVQSGGGVVQPGTSLRLSCAASGFTFSSYGMHWVRQAPGKGLEWVAVISYDGSNKYYADSVKGRFTISRDNSKNTLYLQMNSLRAEDTAVYYCAKDYSYYYGSGSYFNAFDIWGQGTMVTVSS

SEQ ID NO: 54 - protein, 108 aa, synthetic construct
  source 1..108: note = VL of scFv SH1986-E3
  CHAIN 26..31: note = CDR1
  CHAIN 49..51: note = CDR2
  CHAIN 88..98: note = CDR3
SSELTQDPAVSVALGQTVGITCQGDSLRSSFASWYQQKPGQAPILVIYGKNNRPSGIPDRFSGSSSGNTVSLTITGAQAEDEADYYCNSRDSSGNHLVFGGGTKLTVL

SEQ ID NO: 55 - protein, 124 aa, synthetic construct
  source 1..124: note = VH of scFv SH1986-G11
  CHAIN 26..33: note = CDR1
  CHAIN 51..58: note = CDR2
  CHAIN 97..113: note = CDR3
QVQLVQSGAEVEKPGASVKVSCKVSGYTLTKLSMHWVRQAPGKGLEWMGGFDPEDGETIYAQKFQGRVTMTEDTSTDTAYMELSSLRSEDTAVYYCATDILGYCSSTSCYRDYWGQGTLVTVSS

SEQ ID NO: 56 - protein, 112 aa, synthetic construct
  source 1..112: note = VL of scFv SH1986-G11
  CHAIN 27..37: note = CDR1
  CHAIN 55..57: note = CDR2
  CHAIN 94..102: note = CDR3
EVVLTQSPLSLPISLGQPASISCRSSQSLLHSNGYNYLDWYLQKPGQSPQLLIYLGSNRASGVPDRFSGSGSGTDFTLKISRVEAEDVGVYYCMQALQTPRTFGQGTKVEIK

SEQ ID NO: 57 - protein, 119 aa, synthetic construct
  source 1..119: note = VH of scFv VS002-B5
  CHAIN 26..33: note = CDR1
  CHAIN 51..58: note = CDR2
  CHAIN 97..108: note = CDR3
QVQLQQSGAEMKKPGASVKVSCKASGYTFTKYYMHWVRQAPGQGLEWMGIIDPSGGSTSYAQSFQGRVTMTRDTSTTTVYMELTSLRSEDTAVYYCARGGVPGHYFNWWGQGTLVTVSS

SEQ ID NO: 58 - protein, 110 aa, synthetic construct
  source 1..110: note = VL of scFv VS002-B5
  CHAIN 26..31: note = CDR1
  CHAIN 49..51: note = CDR2
  CHAIN 88..100: note = CDR3
QLVLTQSSSVSVAPGKTARITCGGNNIGSKSVHWYQQKPGQAPVLVIYYDSDRPSGIPERFSGSNSGNTATLTISRVEAGDEADYYCQVWDSSSDHPDVVFGGGTKLTVL

SEQ ID NO: 59 - protein, 120 aa, synthetic construct
  source 1..120: note = VH of scFv VS002-C4
  CHAIN 26..33: note = CDR1
  CHAIN 51..60: note = CDR2
  CHAIN 99..109: note = CDR3
QMQLVQSGGGLVQPGGSLRLSCAASGFTFSDYYMDWVRQAPGKGLEWVGRIRNKADSYNIDYAASVTGRFTISRDDSKKSLYLQMNSLKIEDTALYYCARISRFDAFDIWGQGTMVTVSS

SEQ ID NO: 60 - protein, 110 aa, synthetic construct
  source 1..110: note = VL of scFv VS002-C4
  CHAIN 26..33: note = CDR1
  CHAIN 51..53: note = CDR2
  CHAIN 90..100: note = CDR3
QPVLTQPPSASGTPGQRVNISCSGGSSNIGSNHVFWYQQFPGTAPRLVIYRNNQRPSGVPDRFSGSKSGTSASLVISGLRSEDEADYYCAAWDDSLSGWVFGGGTKLTVL

SEQ ID NO: 61 - protein, 118 aa, synthetic construct
  source 1..118: note = VH of scFv VS002-C5
  CHAIN 26..33: note = CDR1
  CHAIN 51..58: note = CDR2
  CHAIN 97..107: note = CDR3
QVQLVQSGGGLVQPGGSLRLSCAASGFTFSSYAMSWVRQAPGKGLEWVSAISGSGGSTYYADSVKGRFTISRDNSKNTLYLQMNSLRAEDTAVYYCARGWQLWGIDYWGQGTLVTVSS

SEQ ID NO: 62 - protein, 112 aa, synthetic construct
  source 1..112: note = VL of scFv VS002-C5
  CHAIN 26..33: note = CDR1
  CHAIN 51..53: note = CDR2
  CHAIN 92..102: note = CDR3
LPVLTQPHSVSGSPGKTVTISCTRSSGSIAGNYVHWYQQRPGSAPTTVIYEDNQRPSGVPDRFSGSIDSSSNSASLTISGLKTEDEADYYCQSYDGDVQHVVFGGGTKVTVL

SEQ ID NO: 63 - protein, 123 aa, synthetic construct
  source 1..123: note = VH of scFv VS002-G9
  CHAIN 26..33: note = CDR1
  CHAIN 51..58: note = CDR2
  CHAIN 97..112: note = CDR3
QVQLVESGGGLVQPGGSLRLSCAASGFTFSSFGMHWVRQAPGKGLEWVSAISGSGGSTYYADSVKGRFTISRDNSKNTLYLQMNSLRAEDTAVYYCAKGAYDYGYYYYGMDVWGQGTTVTVSS

SEQ ID NO: 64 - protein, 110 aa, synthetic construct
  source 1..110: note = VL of scFv VS002-G9
  CHAIN 26..33: note = CDR1
  CHAIN 51..53: note = CDR2
  CA_BIND 92..100: note = CDR3
NFMLTQPHSVSESPGKTVTISCTRSSGSIASNYVQWYQQRPGSAPTTVIYEDNQRPSGVPDRFSGSIDSSSNSASLTISGLKTEDEADYYCQSSDSNIEVFGGGTKLTVL

SEQ ID NO: 65 - protein, 120 aa, synthetic construct
  source 1..120: note = VH of scFv MRU185-3-C11
  CHAIN 26..33: note = CDR1
  CHAIN 51..58: note = CDR2
  CHAIN 97..109: note = CDR3
EVQLVQSGGGVVQPGRSLRLSCAASGFTFSSYAMHWVRQAPGKGLEWVAVISYDGSNKYYADSVKGRFTISRDNSKNTLYLQMNSLRAEDTAVYYCARGFGGATSYFDYWGQGTLVTVSS

SEQ ID NO: 66 - protein, 108 aa, synthetic construct
  source 1..108: note = VL of scFv MRU185-3-C11
  CHAIN 26..31: note = CDR1
  CHAIN 49..51: note = CDR2
  CHAIN 88..98: note = CDR3
SSELTQDPAVSVALGQTVRITCQGDSLRSYYASWYQQKPGRAPVLVIYGKNNRPSGIPDRFSGSSSGNTASLTITGAQAEDEADYYCNSRDSSGNPVVFGGGTKLTVL

SEQ ID NO: 67 - protein, 117 aa, synthetic construct
  source 1..117: note = VH of scFv MRU185-3-E1
  CHAIN 51..58: note = CDR2
  CHAIN 97..106: note = CDR3
  CHAIN 26..33: note = CDR1
QVQLQESGGGVVQPGRSLRLSCAASGFTFSSYGMHWVRQAPGKGLEWVAVISYDGSKKYYADSVKGRFTISRDNAKNTLYLQMNSLRAEDTAVYYCATGNSHAFDIWGQGTMVTVSS

SEQ ID NO: 68 - protein, 107 aa, synthetic construct
  source 1..107: note = VL of scFv MRU185-3-E1
  CHAIN 27..32: note = CDR1
  CHAIN 50..52: note = CDR2
  CHAIN 89..97: note = CDR3
DIQMTQSPSTLTASVGDRVTVTCRASQTINRWLAWYQQKPGKAPKLLIYLASSLDSGVPSRFSGSGSGTEFTLTISSLQPDDFATYYCQQYNAYPRTFGRGTKVEIK